European Patent Specification EP 3 395 329 B1, published April 15, 2026. Title: Preparation Method of Adiposomes, and Use Thereof. Applicant: The Institute of BioPhysics, Chinese Academy of Sciences. Application 16877539.3. The sequence listing filed with the application follows.

SEQUENCE LISTING (14 sequences)

SEQ ID NO: 1 - DNA, 831 bp, Artificial Sequence
  MLDS gene
atgactgaccagaagaccatcgacagcgtcaagacctcgctgtacgcggccgtaggcgccggagacgtcgtcgtgcaggccgtggccgacgtcgtcgcccaggtccgctcgcgcgccgagtccacccagggtgacgtcgaagagcgtgtcggcggcgccaaggagcgcatcgccggactccaggaagaggtcaccgagggtgtcgagaaccttcgcgaccgcctcgccggactgccgtccgagctgcccgaggagcttgccgagctgcgtgagaagttcaccgccgacgagctgcgcaaggttgccgaggcctacctgaaggtcgcctccgacctgtacacgtcgctcgccgagcgcggcgaggacaccgtcgagcgcatccgcaagcagccggtcgtcgaggagggcatcggccgcgccgagaccgccttcggtgacgccgtcgagctgaccgaggaagctctcggcaccgttgcacgccagacgcgcgccgtcggcgagcaggccgcaaagctcgcgggccgcgcttcgggtcgcatctccgacaccgccgagggactcggcgaggccatcgccgacgccggcgacgaggctgccctgaaggttctcgacctgggcgaccaggccgaggaagcgtcgaaggacgctgccgatcgcgtcaccgccaccgcggccgacgtccaggctcgcgccgacaaggctgccccggccaagcacgccgctcccgcgaagaaggctgctccggccaaggctgcggcaaccccggccccggccccggccaagaaggccgccgctccggccaagaaggctgctccggccaagaaggcttga

SEQ ID NO: 2 - protein, 276 aa, Artificial Sequence
  MLDS protein
MTDQKTIDSVKTSLYAAVGAGDVVVQAVADVVAQVRSRAESTQGDVEERVGGAKERIAGLQEEVTEGVENLRDRLAGLPSELPEELAELREKFTADELRKVAEAYLKVASDLYTSLAERGEDTVERIRKQPVVEEGIGRAETAFGDAVELTEEALGTVARQTRAVGEQAAKLAGRASGRISDTAEGLGEAIADAGDEAALKVLDLGDQAEEASKDAADRVTATAADVQARADKAAPAKHAAPAKKAAPAKAAATPAPAPAKKAAAPAKKAAPAKKA

SEQ ID NO: 3 - DNA, 1257 bp, Artificial Sequence
  MDT-28 gene
atgactgacgtcgagcagccagtatcagttgaggatcaacaagcccaagcccaaagctactacgatcaagtcttaggaaatgcttacgtacaaacggcaatcaatgcatacacaaagactaaagagttccatccacttcttaactccacattgaattcagccgaagaaaaggtttccactgtcggaaattatgcggctcaaaaagcctatgacggatacaattcgtactacgttaagccaaagaacaccgcttatgaagcagtctcttatggaaccgagagggccaaaacagctgttgagagcggaaagcaagctgctatcgttggtggtacattcggaattggagctgccgtcgttttgacccaattctcacttgccttgagtgctggaggtgccgccctggtccttgagcaagtggacagtgctaaaaagttgggaagcagcgcgatttctacgatcaaagaagccgagcttgctgtcgaacacagaatcttctcagctcttcatcaggcccaacgaatcgccatggttcctgtggagaaaatcacagaaaatactaattcattgcttgacattcttgacggagcagttcagaaaggactcaatatcgaggtcccaccatctgtgaacctcaccatcggacagcgagtcaaaaatctggcttcactgatcgtccaaggagtatctaacaagctttttaaggcacatgatcatgttatcgatccaatcaacgagagagcccgtaattatcttgagcagctcagccaatccttcgtattgctagacatcgtccgtgagaagaaaacgtgggtcatagagaagtcaaacgagctctccacatctgtctttgatttcaagaaaacacttgaggaagaggcacaaaaatacaaagttgctccagaagagatgttgatgaaacacattcaatcaacctccgagcaactctcaacacaacttcaatcattgcgtgagaagggacaaaacgttttcggtgatggaactaagattgactccaccattgactacttggagaacttgaagaagaacttcacagatgctgaggatgtttacaaagtccgcgacgaggttctgaacgagggacgtcaacggatcgccgagctttcaacctggacgactagccttttgattatctcggccgaatggcaatttgaacctgaagatctactaatcgaagagctctacttcgatgcgccaccgccagttcgcacaagaaacttgtataggaatcgtgcctaa

SEQ ID NO: 4 - protein, 418 aa, Artificial Sequence
  MDT-28 protein
MTDVEQPVSVEDQQAQAQSYYDQVLGNAYVQTAINAYTKTKEFHPLLNSTLNSAEEKVSTVGNYAAQKAYDGYNSYYVKPKNTAYEAVSYGTERAKTAVESGKQAAIVGGTFGIGAAVVLTQFSLALSAGGAALVLEQVDSAKKLGSSAISTIKEAELAVEHRIFSALHQAQRIAMVPVEKITENTNSLLDILDGAVQKGLNIEVPPSVNLTIGQRVKNLASLIVQGVSNKLFKAHDHVIDPINERARNYLEQLSQSFVLLDIVREKKTWVIEKSNELSTSVFDFKKTLEEEAQKYKVAPEEMLMKHIQSTSEQLSTQLQSLREKGQNVFGDGTKIDSTIDYLENLKKNFTDAEDVYKVRDEVLNEGRQRIAELSTWTTSLLIISAEWQFEPEDLLIEELYFDAPPPVRTRNLYRNRA

SEQ ID NO: 5 - DNA, 1314 bp, Artificial Sequence
  Perilipin-2 gene
atggcatccgttgcagttgatccacaaccgagtgtggtgactcgggtggtcaacctgcccttggtgagctccacgtatgacctcatgtcctcagcctatctcagtacaaaggaccagtatccctacctgaagtctgtgtgtgagatggcagagaacggtgtgaagaccatcacctccgtggccatgaccagtgctctgcccatcatccagaagctagagccgcaaattgcagttgccaatacctatgcctgtaaggggctagacaggattgaggagagactgcctattctgaatcagccatcaactcagattgttgccaatgccaaaggcgctgtgactggggcaaaagatgctgtgacgactactgtgactggggccaaggattctgtggccagcacgatcacaggggtgatggacaagaccaaaggggcagtgactggcagtgtggagaagaccaagtctgtggtcagtggcagcattaacacagtcttggggagtcggatgatgcagctcgtgagcagtggcgtagaaaatgcactcaccaaatcagagctgttggtagaacagtacctccctctcactgaggaagaactagaaaaagaagcaaaaaaagttgaaggatttgatctggttcagaagccaagttattatgttagactgggatccctgtctaccaagcttcactcccgtgcctaccagcaggctctcagcagggttaaagaagctaagcaaaaaagccaacagaccatttctcagctccattctactgttcacctgattgaatttgccaggaagaatgtgtatagtgccaatcagaaaattcaggatgctcaggataagctctacctctcatgggtagagtggaaaaggagcattggatatgatgatactgatgagtcccactgtgctgagcacattgagtcacgtactcttgcaattgcccgcaacctgactcagcagctccagaccacgtgccacaccctcctgtccaacatccaaggtgtaccacagaacatccaagatcaagccaagcacatgggggtgatggcaggcgacatctactcagtgttccgcaatgctgcctcctttaaagaagtgtctgacagcctcctcacttctagcaaggggcagctgcagaaaatgaaggaatctttagatgacgtgatggattatcttgttaacaacacgcccctcaactggctggtaggtcccttttatcctcagctgactgagtctcagaatgctcaggaccaaggtgcagagatggacaagagcagccaggagacccagcgatctgagcataaaactcattaa

SEQ ID NO: 6 - protein, 437 aa, Artificial Sequence
  Perilipin-2 protein
MASVAVDPQPSVVTRVVNLPLVSSTYDLMSSAYLSTKDQYPYLKSVCEMAENGVKTITSVAMTSALPIIQKLEPQIAVANTYACKGLDRIEERLPILNQPSTQIVANAKGAVTGAKDAVTTTVTGAKDSVASTITGVMDKTKGAVTGSVEKTKSVVSGSINTVLGSRMMQLVSSGVENALTKSELLVEQYLPLTEEELEKEAKKVEGFDLVQKPSYYVRLGSLSTKLHSRAYQQALSRVKEAKQKSQQTISQLHSTVHLIEFARKNVYSANQKIQDAQDKLYLSWVEWKRSIGYDDTDESHCAEHIESRTLAIARNLTQQLQTTCHTLLSNIQGVPQNIQDQAKHMGVMAGDIYSVFRNAASFKEVSDSLLTSSKGQLQKMKESLDDVMDYLVNNTPLNWLVGPFYPQLTESQNAQDQGAEMDKSSQETQRSEHKTH

SEQ ID NO: 7 - DNA, 1515 bp, Artificial Sequence
  ATGL gene
atgtttccccgcgagaagacgtggaacatctcgttcgcgggctgcggcttcctcggcgtctactacgtcggcgtggcctcctgcctccgcgagcacgcgcccttcctggtggccaacgccacgcacatctacggcgcctcggccggggcgctcacggccacggcgctggtcaccggggtctgcctgggtgaggctggtgccaagttcattgaggtatctaaagaggcccggaagcggttcctgggccccctgcacccctccttcaacctggtaaagatcatccgcagtttcctgctgaaggtcctgcctgctgatagccatgagcatgccagtgggcgcctgggcatctccctgacccgcgtgtcagacggcgagaatgtcattatatcccacttcaactccaaggacgagctcatccaggccaatgtctgcagcggtttcatccccgtgtactgtgggctcatccctccctccctccagggggtgcgctacgtggatggtggcatttcagacaacctgccactctatgagcttaagaacaccatcacagtgtcccccttctcgggcgagagtgacatctgtccgcaggacagctccaccaacatccacgagctgcgggtcaccaacaccagcatccagttcaacctgcgcaacctctaccgcctctccaaggccctcttcccgccggagcccctggtgctgcgagagatgtgcaagcagggataccgggatggcctgcgctttctgcagcggaacggcctcctgaaccggcccaaccccttgctggcgttgccccccgcccgcccccacggcccagaggacaaggaccaggcagtggagagcgcccaagcggaggattactcgcagctgcccggagaagatcacatcctggagcacctgcccgcccggctcaatgaggccctgctggaggcctgcgtggagcccacggacctgctgaccaccctctccaacatgctgcctgtgcgtctggccacggccatgatggtgccctacacgctgccgctggagagcgctctgtccttcaccatccgcttgctggagtggctgcccgacgttcccgaggacatccggtggatgaaggagcagacgggcagcatctgccagtacctggtgatgcgcgccaagaggaagctgggcaggcacctgccctccaggctgccggagcaggtggagctgcgccgcgtccagtcgctgccgtccgtgccgctgtcctgcgccgcctacagagaggcactgcccggctggatgcgcaacaacctctcgctgggggacgcgctggccaagtgggaggagtgccagcgccagctgctgctcggcctcttctgcaccaacgtggccttcccgcccgaagctctgcgcatgcgcgcacccgccgacccggctcccgcccccgcggacccagcatccccgcagcaccagctggccgggcctgcccccttgctgagcacccctgctcccgaggcccggcccgtgatcggggccctggggctgtga

SEQ ID NO: 8 - protein, 504 aa, Artificial Sequence
  ATGL protein
MFPREKTWNISFAGCGFLGVYYVGVASCLREHAPFLVANATHIYGASAGALTATALVTGVCLGEAGAKFIEVSKEARKRFLGPLHPSFNLVKIIRSFLLKVLPADSHEHASGRLGISLTRVSDGENVIISHFNSKDELIQANVCSGFIPVYCGLIPPSLQGVRYVDGGISDNLPLYELKNTITVSPFSGESDICPQDSSTNIHELRVTNTSIQFNLRNLYRLSKALFPPEPLVLREMCKQGYRDGLRFLQRNGLLNRPNPLLALPPARPHGPEDKDQAVESAQAEDYSQLPGEDHILEHLPARLNEALLEACVEPTDLLTTLSNMLPVRLATAMMVPYTLPLESALSFTIRLLEWLPDVPEDIRWMKEQTGSICQYLVMRAKRKLGRHLPSRLPEQVELRRVQSLPSVPLSCAAYREALPGWMRNNLSLGDALAKWEECQRQLLLGLFCTNVAFPPEALRMRAPADPAPAPADPASPQHQLAGPAPLLSTPAPEARPVIGALGL

SEQ ID NO: 9 - DNA, 1563 bp, Artificial Sequence
  MLDS-GFP fusion gene
atgactgaccagaagaccatcgacagcgtcaagacctcgctgtacgcggccgtaggcgccggagacgtcgtcgtgcaggccgtggccgacgtcgtcgcccaggtccgctcgcgcgccgagtccacccagggtgacgtcgaagagcgtgtcggcggcgccaaggagcgcatcgccggactccaggaagaggtcaccgagggtgtcgagaaccttcgcgaccgcctcgccggactgccgtccgagctgcccgaggagcttgccgagctgcgtgagaagttcaccgccgacgagctgcgcaaggttgccgaggcctacctgaaggtcgcctccgacctgtacacgtcgctcgccgagcgcggcgaggacaccgtcgagcgcatccgcaagcagccggtcgtcgaggagggcatcggccgcgccgagaccgccttcggtgacgccgtcgagctgaccgaggaagctctcggcaccgttgcacgccagacgcgcgccgtcggcgagcaggccgcaaagctcgcgggccgcgcttcgggtcgcatctccgacaccgccgagggactcggcgaggccatcgccgacgccggcgacgaggctgccctgaaggttctcgacctgggcgaccaggccgaggaagcgtcgaaggacgctgccgatcgcgtcaccgccaccgcggccgacgtccaggctcgcgccgacaaggctgccccggccaagcacgccgctcccgcgaagaaggctgctccggccaaggctgcggcaaccccggccccggccccggccaagaaggccgccgctccggccaagaaggctgctccggccaagaaggctaagcttgcggccgcaatggtgagcaagggcgaggagctgttcaccggggtggtgcccatcctggtcgagctggacggcgacgtaaacggccacaagttcagcgtgtccggcgagggcgagggcgatgccacctacggcaagctgaccctgaagttcatctgcaccaccggcaagctgcccgtgccctggcccaccctcgtgaccaccctgacctacggcgtgcagtgcttcagccgctaccccgaccacatgaagcagcacgacttcttcaagtccgccatgcccgaaggctacgtccaggagcgcaccatcttcttcaaggacgacggcaactacaagacccgcgccgaggtgaagttcgagggcgacaccctggtgaaccgcatcgagctgaagggcatcgacttcaaggaggacggcaacatcctggggcacaagctggagtacaactacaacagccacaacgtctatatcatggccgacaagcagaagaacggcatcaaggtgaacttcaagatccgccacaacatcgaggacggcagcgtgcagctcgccgaccactaccagcagaacacccccatcggcgacggccccgtgctgctgcccgacaaccactacctgagcacccagtccgccctgagcaaagaccccaacgagaagcgcgatcacatggtcctgctggagttcgtgaccgccgccgggatcactctcggcatggacgagctgtacaagtaa

SEQ ID NO: 10 - protein, 520 aa, Artificial Sequence
  MLDS-GFP fusion protein
MTDQKTIDSVKTSLYAAVGAGDVVVQAVADVVAQVRSRAESTQGDVEERVGGAKERIAGLQEEVTEGVENLRDRLAGLPSELPEELAELREKFTADELRKVAEAYLKVASDLYTSLAERGEDTVERIRKQPVVEEGIGRAETAFGDAVELTEEALGTVARQTRAVGEQAAKLAGRASGRISDTAEGLGEAIADAGDEAALKVLDLGDQAEEASKDAADRVTATAADVQARADKAAPAKHAAPAKKAAPAKAAATPAPAPAKKAAAPAKKAAPAKKAKLAAAMVSKGEELFTGVVPILVELDGDVNGHKFSVSGEGEGDATYGKLTLKFICTTGKLPVPWPTLVTTLTYGVQCFSRYPDHMKQHDFFKSAMPEGYVQERTIFFKDDGNYKTRAEVKFEGDTLVNRIELKGIDFKEDGNILGHKLEYNYNSHNVYIMADKQKNGIKVNFKIRHNIEDGSVQLADHYQQNTPIGDGPVLLPDNHYLSTQSALSKDPNEKRDHMVLLEFVTAAGITLGMDELYK

SEQ ID NO: 11 - DNA, 1980 bp, Artificial Sequence
  MDT-28-GFP fusion gene
atgactgacgtcgagcagccagtatcagttgaggatcaacaagcccaagcccaaagctactacgatcaagtcttaggaaatgcttacgtacaaacggcaatcaatgcatacacaaagactaaagagttccatccacttcttaactccacattgaattcagccgaagaaaaggtttccactgtcggaaattatgcggctcaaaaagcctatgacggatacaattcgtactacgttaagccaaagaacaccgcttatgaagcagtctcttatggaaccgagagggccaaaacagctgttgagagcggaaagcaagctgctatcgttggtggtacattcggaattggagctgccgtcgttttgacccaattctcacttgccttgagtgctggaggtgccgccctggtccttgagcaagtggacagtgctaaaaagttgggaagcagcgcgatttctacgatcaaagaagccgagcttgctgtcgaacacagaatcttctcagctcttcatcaggcccaacgaatcgccatggttcctgtggagaaaatcacagaaaatactaattcattgcttgacattcttgacggagcagttcagaaaggactcaatatcgaggtcccaccatctgtgaacctcaccatcggacagcgagtcaaaaatctggcttcactgatcgtccaaggagtatctaacaaggcacatgatcatgttatcgatccaatcaacgagagagcccgtaattatcttgagcagctcagccaatccttcgtattgctagacatcgtccgtgagaagaaaacgtgggtcatagagaagtcaaacgagctctccacatctgtctttgatttcaagaaaacacttgaggaagaggcacaaaaatacaaagttgctccagaagagatgttgatgaaacacattcaatcaacctccgagcaactctcaacacaacttcaatcattgcgtgagaagggacaaaacgttttcggtgatggaactaagattgactccaccattgactacttggagaacttgaagaagaacttcacagatgctgaggatgtttacaaagtccgcgacgaggttctgaacgagggacgtcaacggatcgccgagctttcaacctggacgactagccttttgattatctcggccgaatggcaatttgaacctgaagatctactaatcgaagagctctacttcgatgcgccaccgccagttcgcacaagaaacttgtataggaatcgtgccaagcttgcggccgcaatggtgagcaagggcgaggagctgttcaccggggtggtgcccatcctggtcgagctggacggcgacgtaaacggccacaagttcagcgtgtccggcgagggcgagggcgatgccacctacggcaagctgaccctgaagttcatctgcaccaccggcaagctgcccgtgccctggcccaccctcgtgaccaccctgacctacggcgtgcagtgcttcagccgctaccccgaccacatgaagcagcacgacttcttcaagtccgccatgcccgaaggctacgtccaggagcgcaccatcttcttcaaggacgacggcaactacaagacccgcgccgaggtgaagttcgagggcgacaccctggtgaaccgcatcgagctgaagggcatcgacttcaaggaggacggcaacatcctggggcacaagctggagtacaactacaacagccacaacgtctatatcatggccgacaagcagaagaacggcatcaaggtgaacttcaagatccgccacaacatcgaggacggcagcgtgcagctcgccgaccactaccagcagaacacccccatcggcgacggccccgtgctgctgcccgacaaccactacctgagcacccagtccgccctgagcaaagaccccaacgagaagcgcgatcacatggtcctgctggagttcgtgaccgccgccgggatcactctcggcatggacgagctgtacaagtaa

SEQ ID NO: 12 - protein, 659 aa, Artificial Sequence
  MDT-28-GFP fuion protein
MTDVEQPVSVEDQQAQAQSYYDQVLGNAYVQTAINAYTKTKEFHPLLNSTLNSAEEKVSTVGNYAAQKAYDGYNSYYVKPKNTAYEAVSYGTERAKTAVESGKQAAIVGGTFGIGAAVVLTQFSLALSAGGAALVLEQVDSAKKLGSSAISTIKEAELAVEHRIFSALHQAQRIAMVPVEKITENTNSLLDILDGAVQKGLNIEVPPSVNLTIGQRVKNLASLIVQGVSNKAHDHVIDPINERARNYLEQLSQSFVLLDIVREKKTWVIEKSNELSTSVFDFKKTLEEEAQKYKVAPEEMLMKHIQSTSEQLSTQLQSLREKGQNVFGDGTKIDSTIDYLENLKKNFTDAEDVYKVRDEVLNEGRQRIAELSTWTTSLLIISAEWQFEPEDLLIEELYFDAPPPVRTRNLYRNRAKLAAAMVSKGEELFTGVVPILVELDGDVNGHKFSVSGEGEGDATYGKLTLKFICTTGKLPVPWPTLVTTLTYGVQCFSRYPDHMKQHDFFKSAMPEGYVQERTIFFKDDGNYKTRAEVKFEGDTLVNRIELKGIDFKEDGNILGHKLEYNYNSHNVYIMADKQKNGIKVNFKIRHNIEDGSVQLADHYQQNTPIGDGPVLLPDNHYLSTQSALSKDPNEKRDHMVLLEFVTAAGITLGMDELYK

SEQ ID NO: 13 - DNA, 2031 bp, Artificial Sequence
  Perilipin-2-GFP fusion gene
atggcatccgttgcagttgatccacaaccgagtgtggtgactcgggtggtcaacctgcccttggtgagctccacgtatgacctcatgtcctcagcctatctcagtacaaaggaccagtatccctacctgaagtctgtgtgtgagatggcagagaacggtgtgaagaccatcacctccgtggccatgaccagtgctctgcccatcatccagaagctagagccgcaaattgcagttgccaatacctatgcctgtaaggggctagacaggattgaggagagactgcctattctgaatcagccatcaactcagattgttgccaatgccaaaggcgctgtgactggggcaaaagatgctgtgacgactactgtgactggggccaaggattctgtggccagcacgatcacaggggtgatggacaagaccaaaggggcagtgactggcagtgtggagaagaccaagtctgtggtcagtggcagcattaacacagtcttggggagtcggatgatgcagctcgtgagcagtggcgtagaaaatgcactcaccaaatcagagctgttggtagaacagtacctccctctcactgaggaagaactagaaaaagaagcaaaaaaagttgaaggatttgatctggttcagaagccaagttattatgttagactgggatccctgtctaccaagcttcactcccgtgcctaccagcaggctctcagcagggttaaagaagctaagcaaaaaagccaacagaccatttctcagctccattctactgttcacctgattgaatttgccaggaagaatgtgtatagtgccaatcagaaaattcaggatgctcaggataagctctacctctcatgggtagagtggaaaaggagcattggatatgatgatactgatgagtcccactgtgctgagcacattgagtcacgtactcttgcaattgcccgcaacctgactcagcagctccagaccacgtgccacaccctcctgtccaacatccaaggtgtaccacagaacatccaagatcaagccaagcacatgggggtgatggcaggcgacatctactcagtgttccgcaatgctgcctcctttaaagaagtgtctgacagcctcctcacttctagcaaggggcagctgcagaaaatgaaggaatctttagatgacgtgatggattatcttgttaacaacacgcccctcaactggctggtaggtcccttttatcctcagctgactgagtctcagaatgctcaggaccaaggtgcagagatggacaagagcagccaggagacccagcgatctgagcataaaactcatatggtgagcaagggcgaggagctgttcaccggggtggtgcccatcctggtcgagctggacggcgacgtaaacggccacaagttcagcgtgtccggcgagggcgagggcgatgccacctacggcaagctgaccctgaagttcatctgcaccaccggcaagctgcccgtgccctggcccaccctcgtgaccaccctgacctacggcgtgcagtgcttcagccgctaccccgaccacatgaagcagcacgacttcttcaagtccgccatgcccgaaggctacgtccaggagcgcaccatcttcttcaaggacgacggcaactacaagacccgcgccgaggtgaagttcgagggcgacaccctggtgaaccgcatcgagctgaagggcatcgacttcaaggaggacggcaacatcctggggcacaagctggagtacaactacaacagccacaacgtctatatcatggccgacaagcagaagaacggcatcaaggtgaacttcaagatccgccacaacatcgaggacggcagcgtgcagctcgccgaccactaccagcagaacacccccatcggcgacggccccgtgctgctgcccgacaaccactacctgagcacccagtccgccctgagcaaagaccccaacgagaagcgcgatcacatggtcctgctggagttcgtgaccgccgccgggatcactctcggcatggacgagctgtacaagtaa

SEQ ID NO: 14 - protein, 676 aa, Artificial Sequence
  Perilipin-2-GFP fusion protein
MASVAVDPQPSVVTRVVNLPLVSSTYDLMSSAYLSTKDQYPYLKSVCEMAENGVKTITSVAMTSALPIIQKLEPQIAVANTYACKGLDRIEERLPILNQPSTQIVANAKGAVTGAKDAVTTTVTGAKDSVASTITGVMDKTKGAVTGSVEKTKSVVSGSINTVLGSRMMQLVSSGVENALTKSELLVEQYLPLTEEELEKEAKKVEGFDLVQKPSYYVRLGSLSTKLHSRAYQQALSRVKEAKQKSQQTISQLHSTVHLIEFARKNVYSANQKIQDAQDKLYLSWVEWKRSIGYDDTDESHCAEHIESRTLAIARNLTQQLQTTCHTLLSNIQGVPQNIQDQAKHMGVMAGDIYSVFRNAASFKEVSDSLLTSSKGQLQKMKESLDDVMDYLVNNTPLNWLVGPFYPQLTESQNAQDQGAEMDKSSQETQRSEHKTHMVSKGEELFTGVVPILVELDGDVNGHKFSVSGEGEGDATYGKLTLKFICTTGKLPVPWPTLVTTLTYGVQCFSRYPDHMKQHDFFKSAMPEGYVQERTIFFKDDGNYKTRAEVKFEGDTLVNRIELKGIDFKEDGNILGHKLEYNYNSHNVYIMADKQKNGIKVNFKIRHNIEDGSVQLADHYQQNTPIGDGPVLLPDNHYLSTQSALSKDPNEKRDHMVLLEFVTAAGITLGMDELYK